European Patent Application EP 4 364 803 A2, published May 8, 2024. Title: VIRAL VECTORS COMPRISING RDH12 CODING REGIONS AND METHODS OF TREATING RETINAL DYSTROPHIES. Applicant: The Regents of the University of Michigan. Application EP. The sequence listing filed with the application follows.

SEQUENCE LISTING (5 sequences)

SEQ ID NO: 1 - DNA, 990 bp, Homo sapiens
  source 1..990: mol_type = genomic DNA
agttggaacgatgctggtcaccttgggactgctcacctccttcttctcgttcctgtatatggtagctccatccatcaggaagttctttgctggtggagtgtgtagaacaaatgtgcagcttcctggcaaggtagtggtgatcactggcgccaacacgggcattggcaaggagacggccagagagctcgctagccgaggagcccgagtctatattgcctgcagagatgtactgaagggggagtctgctgccagtgaaatccgagtggatacaaagaactcccaggtgctggtgcggaaattggacctatccgacaccaaatctatccgagcctttgctgagggctttctggcagaggaaaagcagctccatattctgatcaacaatgcgggagtaatgatgtgtccatattccaagacagctgatggctttgaaacccacctgggagtcaaccacctgggccacttcctcctcacctacctgctcctggagcggctaaaggtgtctgcccctgcacgggtggttaatgtgtcctcggtggctcaccacattggcaagattcccttccacgacctccagagcgagaagcgctacagcaggggttttgcctattgccacagcaagctggccaatgtgctttttactcgtgagctggccaagaggctccaaggcaccggggtcaccacctacgcagtgcacccaggcgtcgtccgctctgagctggtccggcactcctccctgctctgcctgctctggcggctcttctccccctttgtcaagacggcacgggagggggcgcagaccagcctgcactgcgccctggctgagggcctggagcccctgagtggcaagtacttcagtgactgcaagaggacctgggtgtctccaagggcccgaaataacaaaacagctgagcgcctatggaatgtcagctgtgagcttctaggaatccggtgggagtagctggtggaagagctgcagctttatcaggc

SEQ ID NO: 2 - protein, 316 aa, Homo sapiens
MLVTLGLLTSFFSFLYMVAPSIRKFFAGGVCRTNVQLPGKVVVITGANTGIGKETARELASRGARVYIACRDVLKGESAASEIRVDTKNSQVLVRKLDLSDTKSIRAFAEGFLAEEKQLHILINNAGVMMCPYSKTADGFETHLGVNHLGHFLLTYLLLERLKVSAPARVVNVSSVAHHIGKIPFHDLQSEKRYSRGFAYCHSKLANVLFTRELAKRLQGTGVTTYAVHPGVVRSELVRHSSLLCLLWRLFSPFVKTAREGAQTSLHCALAEGLEPLSGKYFSDCKRTWVSPRARNNKTAERLWNVSCELLGIRWE

SEQ ID NO: 3 - DNA, 199 bp, Homo sapiens
  source 1..199: mol_type = genomic DNA
gggccccagaagcctggtggttgtttgtccttctcaggggaaaagtgaggcggccccttggaggaaggggccgggcagaatgatctaatcggattccaagcagctcaggggattgtctttttctagcaccttcttgccactcctaagcgtcctccgtgaccccggctgggatttagcctggtgctgtgtcagccccggt

SEQ ID NO: 4 - protein, 12 aa, Mus musculus
SPFFKSTSQGAQ

SEQ ID NO: 5 - protein, 16 aa, Homo sapiens
DCKRTWVSPRARNNKT